European Patent Specification EP 3 538 673 B1, published May 20, 2026. Title: IDENTIFICATION OF INSTANCE-SPECIFIC SOMATIC GENOME ALTERATIONS WITH FUNCTIONAL IMPACT. Applicant: University of Pittsburgh - Of the Commonwealth System of Higher Education. The sequence listing filed with the application follows.

SEQUENCE LISTING (4 sequences)

SEQ ID NO: 1 - DNA, 25 bp, artificial sequence
  Oligonucleotide priimer
gguauauuacgaagaauugcagagt

SEQ ID NO: 2 - DNA, 25 bp, artificial sequence
  Oligonucleotide primer
acaaauggaggaauacuaacaacag

SEQ ID NO: 3 - DNA, 25 bp, artificial sequence
  Oligonucleotide primer
cgaugcuucagaaacaaaggaagac

SEQ ID NO: 4 - DNA, 25 bp, artificial sequence
  oligonucleotide primer
ggaacgacagagaaauaaagauuca